European Patent Specification EP 3 194 612 B1, published July 3, 2024. Title: METHODS FOR QUANTITATIVE GENETIC ANALYSIS OF CELL FREE DNA. Applicant: Raymond, Christopher K. Kim, Lee P. Armour, Christopher D. Application PCT. The sequence listing filed with the application follows.

SEQUENCE LISTING (562 sequences)

SEQ ID NO: 1 - DNA, 60 bp, Artificial Sequence
  Probe
taaacattggaaaggtttctaattaaccaggagatccaaaagaaagcggttcaagtagca

SEQ ID NO: 2 - DNA, 60 bp, Artificial Sequence
  Probe
gatctcagtttttttggttaactatgtattttggtatatgaagcttctgggttttgcaca

SEQ ID NO: 3 - DNA, 60 bp, Artificial Sequence
  Probe
gacagataagcatacatattaacatggatatatatgtgaatttcattcaaatggttctca

SEQ ID NO: 4 - DNA, 60 bp, Artificial Sequence
  Probe
agctcttagcctttggggggatgacactcttgagcggacgtggggacgcctcgctcttta

SEQ ID NO: 5 - DNA, 60 bp, Artificial Sequence
  Probe
aagcccccaccgccgcctctttccaaaataaacaccagccagccgccgagcccggagtcg

SEQ ID NO: 6 - DNA, 60 bp, Artificial Sequence
  Probe
gcctcccttccccctccccgcccgacagcggccgctcgggccccggctctcggttataag

SEQ ID NO: 7 - DNA, 60 bp, Artificial Sequence
  Probe
ggtgtggcagccaggggggcgcactctgctctggctgggccccttctcccatgttttctt

SEQ ID NO: 8 - DNA, 60 bp, Artificial Sequence
  Probe
ttacacaacctttgggcttggacaacactttggggtccaaagaacctaagagtctttctg

SEQ ID NO: 9 - DNA, 60 bp, Artificial Sequence
  Probe
tgatgaaacttgggctggatggggcacaggtagggtgcttgttgctttcagtcagatgaa

SEQ ID NO: 10 - DNA, 60 bp, Artificial Sequence
  Probe
aatgaaagaaaaggaggccagattgctactcctggtccctgccacacactaggtacccta

SEQ ID NO: 11 - DNA, 60 bp, Artificial Sequence
  Probe
attgacaatacctacataaaactctttccagaatgttgttaagtcttagtcattagggag

SEQ ID NO: 12 - DNA, 60 bp, Artificial Sequence
  Probe
ggatttccaccaacactgtattcatgtacccatttttctcttaacctaactttattggtc

SEQ ID NO: 13 - DNA, 60 bp, Artificial Sequence
  Probe
caaagggggaaaaccatcaggacattatttaacaacggaaatatctaactgaaaggcaaa

SEQ ID NO: 14 - DNA, 60 bp, Artificial Sequence
  Probe
caggcagaccaaccaaagtctttgttccaccttttaaaactaaatcacattttcacagag

SEQ ID NO: 15 - DNA, 60 bp, Artificial Sequence
  Probe
ccccagccagcggtccgcaacccttgccgcatccacgaaactttgcccatagcagcgggc

SEQ ID NO: 16 - DNA, 60 bp, Artificial Sequence
  Probe
cgactcatctcagcattaaagtgataaaaaaataaattaaaaggcaagtggacttcggtg

SEQ ID NO: 17 - DNA, 60 bp, Artificial Sequence
  Probe
ctgtggcgcgcactgcgcgctgcgccaggtttccgcaccaagacccctttaactcaagac

SEQ ID NO: 18 - DNA, 60 bp, Artificial Sequence
  Probe
ttctactgcgacgaggaggagaacttctaccagcagcagcagcagagcgagctgcagccc

SEQ ID NO: 19 - DNA, 60 bp, Artificial Sequence
  Probe
accgagctgctgggaggagacatggtgaaccagagtttcatctgcgacccggacgacgag

SEQ ID NO: 20 - DNA, 60 bp, Artificial Sequence
  Probe
gccgccgcctcagagtgcatcgacccctcggtggtcttcccctaccctctcaacgacagc

SEQ ID NO: 21 - DNA, 60 bp, Artificial Sequence
  Probe
ggcggctaggggacaggggcggggtgggcagcagctcgaatttcttccagatatcctcgc

SEQ ID NO: 22 - DNA, 60 bp, Artificial Sequence
  Probe
agacgagcttggcggcggccgagaagccgctccacatacagtcctggatgatgatgtttt

SEQ ID NO: 23 - DNA, 60 bp, Artificial Sequence
  Probe
aggagagcagagaatccgaggacggagagaaggcgctggagtcttgcgaggcgcaggact

SEQ ID NO: 24 - DNA, 60 bp, Artificial Sequence
  Probe
taagagtggcccgttaaataagctgccaatgaaaatgggaaaggtatccagccgcccact

SEQ ID NO: 25 - DNA, 60 bp, Artificial Sequence
  Probe
ttgtatttgtacagcattaatctggtaattgattattttaatgtaaccttgctaaaggag

SEQ ID NO: 26 - DNA, 60 bp, Artificial Sequence
  Probe
gaggccacagcaaacctcctcacagcccactggtcctcaagaggtgccacgtctccacac

SEQ ID NO: 27 - DNA, 60 bp, Artificial Sequence
  Probe
agaggaggaacgagctaaaacggagcttttttgccctgcgtgaccagatcccggagttgg

SEQ ID NO: 28 - DNA, 60 bp, Artificial Sequence
  Probe
tccaacttgaccctcttggcagcaggatagtccttccgagtggagggaggcgctgcgtag

SEQ ID NO: 29 - DNA, 60 bp, Artificial Sequence
  Probe
gcttggacggacaggatgtatgctgtggcttttttaaggataactaccttgggggccttt

SEQ ID NO: 30 - DNA, 60 bp, Artificial Sequence
  Probe
gcatttgatcatgcatttgaaacaagttcataggtgattgctcaggacatttctgttaga

SEQ ID NO: 31 - DNA, 60 bp, Artificial Sequence
  Probe
cgccccgcgccctcccagccgggtccagccggagccatggggccggagccgcagtgagca

SEQ ID NO: 32 - DNA, 60 bp, Artificial Sequence
  Probe
ctctggccccgccggccgcgggacctcggcggggcatccacagggcagggtcccgccgct

SEQ ID NO: 33 - DNA, 60 bp, Artificial Sequence
  Probe
ggcatgacttggagtgagtttggatggggtggccaggtctgagaaggtcccccgccagtg

SEQ ID NO: 34 - DNA, 60 bp, Artificial Sequence
  Probe
gcagggcaccttcttctgccacccacctgtaaacagagggctcagcccagctggaggcag

SEQ ID NO: 35 - DNA, 60 bp, Artificial Sequence
  Probe
cccaagatctccaagtactggggaaccccagggaggccctggggggtggcagtgttccta

SEQ ID NO: 36 - DNA, 60 bp, Artificial Sequence
  Probe
ctaatgcacacaaagcctccccctggttagcagtggccctggtcagctctgaataaccaa

SEQ ID NO: 37 - DNA, 60 bp, Artificial Sequence
  Probe
ctgctcctcttttagaaggcaggagggccccaagggaagcagaaggtgacagaaggggaa

SEQ ID NO: 38 - DNA, 60 bp, Artificial Sequence
  Probe
tggggcagtggcgggcaggcactgggttgtaagttgggagtttgcggctggggtcaggct

SEQ ID NO: 39 - DNA, 60 bp, Artificial Sequence
  Probe
tctgctgctgtttgtgcctctctctgttactaacccgtcctctcgctgttagacatctct

SEQ ID NO: 40 - DNA, 60 bp, Artificial Sequence
  Probe
cccacccctcccatgtcacctgtatgacacctgcattccacccggccccagccctcccct

SEQ ID NO: 41 - DNA, 60 bp, Artificial Sequence
  Probe
tgggccaggtagtctccctagaaggtgatgctgatgagggtctggtgcccagggcgccac

SEQ ID NO: 42 - DNA, 60 bp, Artificial Sequence
  Probe
ggtgcccaccccttgcatcctggggggtagagcacattgggcacaaagcagaggcacata

SEQ ID NO: 43 - DNA, 60 bp, Artificial Sequence
  Probe
caccctgcctggtactgccctattgcccctggcacaccagggcaaaacagcacagtgaaa

SEQ ID NO: 44 - DNA, 60 bp, Artificial Sequence
  Probe
ccatttacagaaacaaacctccccaccaaaatgagaaaactgtgtttctccctggcactc

SEQ ID NO: 45 - DNA, 60 bp, Artificial Sequence
  Probe
ttattcttcttgtgcctgggcacggtaatgctgctcatggtggtgcacgaagggccaggg

SEQ ID NO: 46 - DNA, 60 bp, Artificial Sequence
  Probe
gaaggataggacagggtgggctgggccaggctgcatgcgcagagggacaggaactgcagc

SEQ ID NO: 47 - DNA, 60 bp, Artificial Sequence
  Probe
gggcccggaccctgatgctcatgtggctgttgacctgtcccggtatgaaggctgagacgg

SEQ ID NO: 48 - DNA, 60 bp, Artificial Sequence
  Probe
tctgtctcctgccatccccaagagatgctgccacatctggatcctcaggactctgtctgc

SEQ ID NO: 49 - DNA, 60 bp, Artificial Sequence
  Probe
tcacgtcccagggcagttttcttccctgaagaaagttggatggcatgatctgtcttccca

SEQ ID NO: 50 - DNA, 60 bp, Artificial Sequence
  Probe
gtgttgagaacagactactgacttctaatagcagcgacttctttaccttgataaaccaca

SEQ ID NO: 51 - DNA, 60 bp, Artificial Sequence
  Probe
aaaaaaaggatgggttccatatgggtggtgtcaagtgcccacctcctagcaagtcagcag

SEQ ID NO: 52 - DNA, 60 bp, Artificial Sequence
  Probe
ccctcacaaggtcaaagctatacatcagctcctgtgacattgactcatcccccagacctt

SEQ ID NO: 53 - DNA, 60 bp, Artificial Sequence
  Probe
aacccaccgagatctgcaaactttgcaggatgcaccagatgtcttgtagccatgggtcaa

SEQ ID NO: 54 - DNA, 60 bp, Artificial Sequence
  TYMSr4r probe
tgcctccctcaggtgcctctgcacaaaaccagattgcttccctctaagagtatggttagt

SEQ ID NO: 55 - DNA, 60 bp, Artificial Sequence
  Probe
gttttactttgcctttagctgtggtctttcaaaccaccatccctccttatcttcctctgc

SEQ ID NO: 56 - DNA, 60 bp, Artificial Sequence
  Probe
ctctgcaatttgttttcccatattaaagaactgaagagctcagtgtggtaggctggcaag

SEQ ID NO: 57 - DNA, 60 bp, Artificial Sequence
  Probe
ttttaaatgatgttttaaagaattgaaactaacatactgttctgctttctcccccgggtt

SEQ ID NO: 58 - DNA, 60 bp, Artificial Sequence
  Probe
cctgcccaccacttctccctaaactgaagccccacatttggagcagtcatctttatcttg

SEQ ID NO: 59 - DNA, 60 bp, Artificial Sequence
  Probe
ggttgcgctccaatcatgttacataacctacggcaaggtatcgacaggatcatactcctg

SEQ ID NO: 60 - DNA, 60 bp, Artificial Sequence
  Probe
gcacagttacatttgccagtggcaacatccttaaaaattaataactgataggtcacggac

SEQ ID NO: 61 - DNA, 60 bp, Artificial Sequence
  Probe
cgtcccgccgcgccacttggcctgcctccgtcccgccgcgccacttcgcctgcctccgtc

SEQ ID NO: 62 - DNA, 60 bp, Artificial Sequence
  Probe
ctgtaaggcgaggaggacgatgcgtcccctccctcgcaggattgaggttaggactaaacg

SEQ ID NO: 63 - DNA, 35 bp, Artificial Sequence
  Partner Oligo #138
gtgaaaaccaggatcaactcccgtgccagtcacat

SEQ ID NO: 64 - DNA, 20 bp, Artificial Sequence
  Adaptor
  misc_feature (1)..(8): n is a, c, g, or t
nnnnnnnncatggccgcagg

SEQ ID NO: 65 - DNA, 20 bp, Artificial Sequence
  Adaptor
  misc_feature (1)..(8): n is a, c, g, or t
nnnnnnnnatcttagtggca

SEQ ID NO: 66 - DNA, 20 bp, Artificial Sequence
  Adaptor
  misc_feature (1)..(8): n is a, c, g, or t
nnnnnnnncggaactcggag

SEQ ID NO: 67 - DNA, 20 bp, Artificial Sequence
  Adaptor
  misc_feature (1)..(8): n is a, c, g, or t
nnnnnnnngactccgatccc

SEQ ID NO: 68 - DNA, 95 bp, Artificial Sequence
  Probe
atgtgactggcacgggagttgatcctggttttcacgggtttgagtggcatgagctacctactggatgtgcctgactgtttccccttcttcttccc

SEQ ID NO: 69 - DNA, 95 bp, Artificial Sequence
  Probe
atgtgactggcacgggagttgatcctggttttcacctatctccaggatggagagagggaaaaaaaagatgggtctgtgtgggagggcaggtactt

SEQ ID NO: 70 - DNA, 95 bp, Artificial Sequence
  Probe
atgtgactggcacgggagttgatcctggttttcacgaaagaagccaggtcttcaattaataagattccctggtctcgtttgtctacctgttaatg

SEQ ID NO: 71 - DNA, 95 bp, Artificial Sequence
  Probe
atgtgactggcacgggagttgatcctggttttcaccagactcgcgcccaattttcccccaccccttgttattgccacaaaatcctgaggatgatc

SEQ ID NO: 72 - DNA, 95 bp, Artificial Sequence
  Probe
atgtgactggcacgggagttgatcctggttttcacaagcacctagccccattcctgctgagcaggaggtggcaggtaccccagactgggaggtaa

SEQ ID NO: 73 - DNA, 95 bp, Artificial Sequence
  Probe
atgtgactggcacgggagttgatcctggttttcacagtcggtggggccaggatgaggcccagtctgttcacacatggctgctgcctctcagctct

SEQ ID NO: 74 - DNA, 95 bp, Artificial Sequence
  Probe
atgtgactggcacgggagttgatcctggttttcaccctggccctcagccagtacagaaagtcatttgtcaaggccttcagttggcagacgtgctc

SEQ ID NO: 75 - DNA, 95 bp, Artificial Sequence
  Probe
atgtgactggcacgggagttgatcctggttttcacagaattcattgccagctataaatctgtggaaacgctgccacacaatcttagcacacaaga

SEQ ID NO: 76 - DNA, 95 bp, Artificial Sequence
  Probe
atgtgactggcacgggagttgatcctggttttcacttacttccctccagttttgttgcttgcaaaacaacagaatcttctctccatgaaatcatg

SEQ ID NO: 77 - DNA, 95 bp, Artificial Sequence
  Probe
atgtgactggcacgggagttgatcctggttttcaccaggggtatctattatccccattttctcacaaaggaaaccaagataaaaggtttaaatgg

SEQ ID NO: 78 - DNA, 95 bp, Artificial Sequence
  Probe
atgtgactggcacgggagttgatcctggttttcactgttacctttaaaagacatctgctttctgccaaaattaatgtgctgaacttaaacttacc

SEQ ID NO: 79 - DNA, 95 bp, Artificial Sequence
  Probe
atgtgactggcacgggagttgatcctggttttcacttcccagtaaattactcttaccaatgcaacagactttaaagaagttgtgttttacaatgc

SEQ ID NO: 80 - DNA, 95 bp, Artificial Sequence
  Probe
atgtgactggcacgggagttgatcctggttttcactaaatgacataacagttatgattttgcagaaaacagatctgtatttatttcagtgttact

SEQ ID NO: 81 - DNA, 95 bp, Artificial Sequence
  Probe
atgtgactggcacgggagttgatcctggttttcacgacaggttttgaaagatatttgtgttactaatgactgtgctataacttttttttctttcc

SEQ ID NO: 82 - DNA, 95 bp, Artificial Sequence
  Probe
atgtgactggcacgggagttgatcctggttttcacctgtggcgcgcactgcgcgctgcgccaggtttccgcaccaagacccctttaactcaagac

SEQ ID NO: 83 - DNA, 95 bp, Artificial Sequence
  Probe
atgtgactggcacgggagttgatcctggttttcacggcggctaggggacaggggcggggtgggcagcagctcgaatttcttccagatatcctcgc

SEQ ID NO: 84 - DNA, 95 bp, Artificial Sequence
  Probe
atgtgactggcacgggagttgatcctggttttcacaccgagctgctgggaggagacatggtgaaccagagtttcatctgcgacccggacgacgag

SEQ ID NO: 85 - DNA, 95 bp, Artificial Sequence
  Probe
atgtgactggcacgggagttgatcctggttttcacaggagagcagagaatccgaggacggagagaaggcgctggagtcttgcgaggcgcaggact

SEQ ID NO: 86 - DNA, 95 bp, Artificial Sequence
  Probe
atgtgactggcacgggagttgatcctggttttcacctgtaagttatcgtaaaaaggagcatctaggtaggtctttgtagccaatgttacccgatt

SEQ ID NO: 87 - DNA, 95 bp, Artificial Sequence
  Probe
atgtgactggcacgggagttgatcctggttttcacaatggccattcttccaggaggcacagaaattacaggccatgcacagagagaaatacccga

SEQ ID NO: 88 - DNA, 95 bp, Artificial Sequence
  Probe
atgtgactggcacgggagttgatcctggttttcaccttgttcgttccttgtactgagaccctagtctgccactgaggatttggtttttgcccttc

SEQ ID NO: 89 - DNA, 95 bp, Artificial Sequence
  Probe
atgtgactggcacgggagttgatcctggttttcacatcaagactcatcagtaccatcaaaagctgagatgaaacagtgtaagtttcaacagaaat

SEQ ID NO: 90 - DNA, 95 bp, Artificial Sequence
  Probe
atgtgactggcacgggagttgatcctggttttcactgtgtccagctgtgaaactcagagatgtaactgctgacatcctccctattttgcatctca

SEQ ID NO: 91 - DNA, 95 bp, Artificial Sequence
  Probe
atgtgactggcacgggagttgatcctggttttcacatttgaaacaattttatcatgaatgccatgaccaaagtattcttctgtatcttctttctt

SEQ ID NO: 92 - DNA, 95 bp, Artificial Sequence
  Probe
atgtgactggcacgggagttgatcctggttttcactgatgggtgggctcccgaaggggcctcccgcagacttgcgaagttcccactctctgggcg

SEQ ID NO: 93 - DNA, 95 bp, Artificial Sequence
  Probe
atgtgactggcacgggagttgatcctggttttcaccagggtgcgggggcatccaggctgcccaagcggaggctgggccggctgtgctggcctctt

SEQ ID NO: 94 - DNA, 95 bp, Artificial Sequence
  Probe
atgtgactggcacgggagttgatcctggttttcacttttgaaatgtgggtttgttgccatgaaacgtgtttcaagcatagttttgacagataacg

SEQ ID NO: 95 - DNA, 95 bp, Artificial Sequence
  Probe
atgtgactggcacgggagttgatcctggttttcactgccctaaaagtgtatgtataacatccctgatgtctgcatttgtcctttgactggtgttt

SEQ ID NO: 96 - DNA, 95 bp, Artificial Sequence
  Probe
atgtgactggcacgggagttgatcctggttttcacaacccctcgaggctcagacctttggagcaggagtgtgattctggccaaccaccctctctg

SEQ ID NO: 97 - DNA, 95 bp, Artificial Sequence
  Probe
atgtgactggcacgggagttgatcctggttttcaccataaatatgtgtgctagtcctgttagacccaagtgctgcccaagggcagcgccctgctc

SEQ ID NO: 98 - DNA, 95 bp, Artificial Sequence
  Probe
atgtgactggcacgggagttgatcctggttttcactacttgttaattaaaaattcaagagtttttttttcttattctgaggttatctttttacca

SEQ ID NO: 99 - DNA, 95 bp, Artificial Sequence
  Probe
atgtgactggcacgggagttgatcctggttttcacccaaaatctgttttccaataaattctcagatccaggaagaggaaaggaaaaacatcaaaa

SEQ ID NO: 100 - DNA, 95 bp, Artificial Sequence
  Probe
atgtgactggcacgggagttgatcctggttttcacatactccatctcccgtaaaaatagtgagacttgagtaatgtttgatgtcacttgtctttc

SEQ ID NO: 101 - DNA, 95 bp, Artificial Sequence
  Probe
atgtgactggcacgggagttgatcctggttttcaccagtcaccactatattattctaggtatcccagaaaagttaaagtcaaatctgaaacacat

SEQ ID NO: 102 - DNA, 95 bp, Artificial Sequence
  Probe
atgtgactggcacgggagttgatcctggttttcaccgccccgcgtccgacccgcggatcccgcggcgtccggcccgggtggtctggatcgcggag

SEQ ID NO: 103 - DNA, 95 bp, Artificial Sequence
  Probe
atgtgactggcacgggagttgatcctggttttcacccatacgggcagcacgacgcgcggactgcgattgcagaagatgacctgggagggctcgcg

SEQ ID NO: 104 - DNA, 95 bp, Artificial Sequence
  Probe
atgtgactggcacgggagttgatcctggttttcactagaggggcttcagaccgtgctatcgtccctgctgggtcgggcctaagcgccgggcccgt

SEQ ID NO: 105 - DNA, 95 bp, Artificial Sequence
  Probe
atgtgactggcacgggagttgatcctggttttcacggcgccgaggaggagatggaggccgggcggccgcggcccgtgctgcgctcggtgaactcg

SEQ ID NO: 106 - DNA, 95 bp, Artificial Sequence
  Probe
atgtgactggcacgggagttgatcctggttttcacggtgtgggccaccgtgcccagccaccggtgtggctctttaacaacctttgcttgtcccga

SEQ ID NO: 107 - DNA, 95 bp, Artificial Sequence
  Probe
atgtgactggcacgggagttgatcctggttttcacaagtggtctatcctgtacttaccacaacaaccttatctttttaaaaagtaaaacgtcagt

SEQ ID NO: 108 - DNA, 95 bp, Artificial Sequence; identical to SEQ ID NO: 88
  Probe

SEQ ID NO: 109 - DNA, 95 bp, Artificial Sequence; identical to SEQ ID NO: 89
  Probe

SEQ ID NO: 110 - DNA, 75 bp, Artificial Sequence
  Probe
atgtgactggcacgggagttgatcctggttttcacacctactggatgtgcctgactgtttccccttcttcttccc

SEQ ID NO: 111 - DNA, 75 bp, Artificial Sequence
  Probe
atgtgactggcacgggagttgatcctggttttcacgggaaaaaaaagatgggtctgtgtgggagggcaggtactt

SEQ ID NO: 112 - DNA, 75 bp, Artificial Sequence
  Probe
atgtgactggcacgggagttgatcctggttttcacttaataagattccctggtctcgtttgtctacctgttaatg

SEQ ID NO: 113 - DNA, 75 bp, Artificial Sequence
  Probe
atgtgactggcacgggagttgatcctggttttcacccccaccccttgttattgccacaaaatcctgaggatgatc

SEQ ID NO: 114 - DNA, 75 bp, Artificial Sequence
  Probe
atgtgactggcacgggagttgatcctggttttcacgctgagcaggaggtggcaggtaccccagactgggaggtaa

SEQ ID NO: 115 - DNA, 75 bp, Artificial Sequence
  Probe
atgtgactggcacgggagttgatcctggttttcacggcccagtctgttcacacatggctgctgcctctcagctct

SEQ ID NO: 116 - DNA, 75 bp, Artificial Sequence
  Probe
atgtgactggcacgggagttgatcctggttttcacgaaagtcatttgtcaaggccttcagttggcagacgtgctc

SEQ ID NO: 117 - DNA, 75 bp, Artificial Sequence
  Probe
atgtgactggcacgggagttgatcctggttttcacaatctgtggaaacgctgccacacaatcttagcacacaaga

SEQ ID NO: 118 - DNA, 75 bp, Artificial Sequence
  Probe
atgtgactggcacgggagttgatcctggttttcactgcttgcaaaacaacagaatcttctctccatgaaatcatg

SEQ ID NO: 119 - DNA, 75 bp, Artificial Sequence
  Probe
atgtgactggcacgggagttgatcctggttttcacattttctcacaaaggaaaccaagataaaaggtttaaatgg

SEQ ID NO: 120 - DNA, 75 bp, Artificial Sequence
  Probe
atgtgactggcacgggagttgatcctggttttcactgctttctgccaaaattaatgtgctgaacttaaacttacc

SEQ ID NO: 121 - DNA, 75 bp, Artificial Sequence
  Probe
atgtgactggcacgggagttgatcctggttttcacccaatgcaacagactttaaagaagttgtgttttacaatgc

SEQ ID NO: 122 - DNA, 75 bp, Artificial Sequence
  Probe
atgtgactggcacgggagttgatcctggttttcacattttgcagaaaacagatctgtatttatttcagtgttact

SEQ ID NO: 123 - DNA, 75 bp, Artificial Sequence
  Probe
atgtgactggcacgggagttgatcctggttttcactgtgttactaatgactgtgctataacttttttttctttcc

SEQ ID NO: 124 - DNA, 75 bp, Artificial Sequence
  Probe
atgtgactggcacgggagttgatcctggttttcactgcgccaggtttccgcaccaagacccctttaactcaagac

SEQ ID NO: 125 - DNA, 75 bp, Artificial Sequence
  Probe
atgtgactggcacgggagttgatcctggttttcacggggtgggcagcagctcgaatttcttccagatatcctcgc

SEQ ID NO: 126 - DNA, 75 bp, Artificial Sequence
  Probe
atgtgactggcacgggagttgatcctggttttcaccatggtgaaccagagtttcatctgcgacccggacgacgag

SEQ ID NO: 127 - DNA, 75 bp, Artificial Sequence
  Probe
atgtgactggcacgggagttgatcctggttttcacgacggagagaaggcgctggagtcttgcgaggcgcaggact

SEQ ID NO: 128 - DNA, 75 bp, Artificial Sequence
  Probe
atgtgactggcacgggagttgatcctggttttcacgagcatctaggtaggtctttgtagccaatgttacccgatt

SEQ ID NO: 129 - DNA, 75 bp, Artificial Sequence
  Probe
atgtgactggcacgggagttgatcctggttttcacgcacagaaattacaggccatgcacagagagaaatacccga

SEQ ID NO: 130 - DNA, 75 bp, Artificial Sequence
  Probe
atgtgactggcacgggagttgatcctggttttcacagaccctagtctgccactgaggatttggtttttgcccttc

SEQ ID NO: 131 - DNA, 75 bp, Artificial Sequence
  Probe
atgtgactggcacgggagttgatcctggttttcactcaaaagctgagatgaaacagtgtaagtttcaacagaaat

SEQ ID NO: 132 - DNA, 75 bp, Artificial Sequence
  Probe
atgtgactggcacgggagttgatcctggttttcacagagatgtaactgctgacatcctccctattttgcatctca

SEQ ID NO: 133 - DNA, 75 bp, Artificial Sequence
  Probe
atgtgactggcacgggagttgatcctggttttcacgaatgccatgaccaaagtattcttctgtatcttctttctt

SEQ ID NO: 134 - DNA, 75 bp, Artificial Sequence
  Probe
atgtgactggcacgggagttgatcctggttttcacgggcctcccgcagacttgcgaagttcccactctctgggcg

SEQ ID NO: 135 - DNA, 75 bp, Artificial Sequence
  Probe
atgtgactggcacgggagttgatcctggttttcacgctgcccaagcggaggctgggccggctgtgctggcctctt

SEQ ID NO: 136 - DNA, 75 bp, Artificial Sequence
  Probe
atgtgactggcacgggagttgatcctggttttcacgccatgaaacgtgtttcaagcatagttttgacagataacg

SEQ ID NO: 137 - DNA, 75 bp, Artificial Sequence
  Probe
atgtgactggcacgggagttgatcctggttttcacaacatccctgatgtctgcatttgtcctttgactggtgttt

SEQ ID NO: 138 - DNA, 75 bp, Artificial Sequence
  Probe
atgtgactggcacgggagttgatcctggttttcactttggagcaggagtgtgattctggccaaccaccctctctg

SEQ ID NO: 139 - DNA, 75 bp, Artificial Sequence
  Probe
atgtgactggcacgggagttgatcctggttttcacctgttagacccaagtgctgcccaagggcagcgccctgctc

SEQ ID NO: 140 - DNA, 75 bp, Artificial Sequence
  Probe
atgtgactggcacgggagttgatcctggttttcacaagagtttttttttcttattctgaggttatctttttacca

SEQ ID NO: 141 - DNA, 75 bp, Artificial Sequence
  Probe
atgtgactggcacgggagttgatcctggttttcacaattctcagatccaggaagaggaaaggaaaaacatcaaaa

SEQ ID NO: 142 - DNA, 75 bp, Artificial Sequence
  Probe
atgtgactggcacgggagttgatcctggttttcacatagtgagacttgagtaatgtttgatgtcacttgtctttc

SEQ ID NO: 143 - DNA, 75 bp, Artificial Sequence
  Probe
atgtgactggcacgggagttgatcctggttttcactaggtatcccagaaaagttaaagtcaaatctgaaacacat

SEQ ID NO: 144 - DNA, 75 bp, Artificial Sequence
  Probe
atgtgactggcacgggagttgatcctggttttcacgatcccgcggcgtccggcccgggtggtctggatcgcggag

SEQ ID NO: 145 - DNA, 75 bp, Artificial Sequence
  Probe
atgtgactggcacgggagttgatcctggttttcacgcggactgcgattgcagaagatgacctgggagggctcgcg

SEQ ID NO: 146 - DNA, 75 bp, Artificial Sequence
  Probe
atgtgactggcacgggagttgatcctggttttcacctatcgtccctgctgggtcgggcctaagcgccgggcccgt

SEQ ID NO: 147 - DNA, 75 bp, Artificial Sequence
  Probe
atgtgactggcacgggagttgatcctggttttcacggccgggcggccgcggcccgtgctgcgctcggtgaactcg

SEQ ID NO: 148 - DNA, 75 bp, Artificial Sequence
  Probe
atgtgactggcacgggagttgatcctggttttcacgccaccggtgtggctctttaacaacctttgcttgtcccga

SEQ ID NO: 149 - DNA, 75 bp, Artificial Sequence
  Probe
atgtgactggcacgggagttgatcctggttttcacaccacaacaaccttatctttttaaaaagtaaaacgtcagt

SEQ ID NO: 150 - DNA, 75 bp, Artificial Sequence; identical to SEQ ID NO: 130
  Probe

SEQ ID NO: 151 - DNA, 75 bp, Artificial Sequence; identical to SEQ ID NO: 131
  Probe

SEQ ID NO: 152 - DNA, 58 bp, Artificial Sequence
  ACA2_FLFP primer
aatgatacggcgaccaccgagatctacacgtcatgcaggaccagagaattcgaataca

SEQ ID NO: 153 - DNA, 57 bp, Artificial Sequence
  CAC3_FLRP primer
caagcagaagacggcatacgagatgtgactggcacgggagttgatcctggttttcac

SEQ ID NO: 154 - DNA, 75 bp, Artificial Sequence
  Probe
atgtgactggcacgggagttgatcctggttttcaccgaatgagggtgatgtttttccgcggcacctccttcaggt

SEQ ID NO: 155 - DNA, 75 bp, Artificial Sequence
  Probe
atgtgactggcacgggagttgatcctggttttcacgttgtagtcggtcatgatggtcgaggtgcggagcttgctc

SEQ ID NO: 156 - DNA, 75 bp, Artificial Sequence
  Probe
atgtgactggcacgggagttgatcctggttttcacgcagctcctggtgcttccggcggtacactgcaggtgggtg

SEQ ID NO: 157 - DNA, 75 bp, Artificial Sequence
  Probe
atgtgactggcacgggagttgatcctggttttcacctacacaggccacttcctacaggaagcctccctggatctc

SEQ ID NO: 158 - DNA, 75 bp, Artificial Sequence
  Probe
atgtgactggcacgggagttgatcctggttttcacgaaatactaataaaatgattaaagaaggtgtgtctttaat

SEQ ID NO: 159 - DNA, 75 bp, Artificial Sequence
  Probe
atgtgactggcacgggagttgatcctggttttcactatatggaaaataattatttgtattatatagggcagagtc

SEQ ID NO: 160 - DNA, 75 bp, Artificial Sequence
  Probe
atgtgactggcacgggagttgatcctggttttcacattagacccaatatggtctgcagattttattagaagaaat

SEQ ID NO: 161 - DNA, 75 bp, Artificial Sequence
  Probe
atgtgactggcacgggagttgatcctggttttcacgtgaaccagcagactgtgttgcaagtataaccccacgtga

SEQ ID NO: 162 - DNA, 75 bp, Artificial Sequence
  Probe
atgtgactggcacgggagttgatcctggttttcacgccatggagcctaaggaagtttcagcaaggccctaagggg

SEQ ID NO: 163 - DNA, 75 bp, Artificial Sequence
  Probe
atgtgactggcacgggagttgatcctggttttcaccccaggaattggcctgccttagtatttctgctgtgctcag

SEQ ID NO: 164 - DNA, 75 bp, Artificial Sequence
  Probe
atgtgactggcacgggagttgatcctggttttcactttgagggtgcagctgggatcttggtcagttgtgtttcct

SEQ ID NO: 165 - DNA, 75 bp, Artificial Sequence
  Probe
atgtgactggcacgggagttgatcctggttttcaccacatcatgaaaagatctctgaattggtgtctggggatct

SEQ ID NO: 166 - DNA, 75 bp, Artificial Sequence
  Probe
atgtgactggcacgggagttgatcctggttttcactgaggaccaggtcacaggacctctttggactgcagtttcc

SEQ ID NO: 167 - DNA, 75 bp, Artificial Sequence
  Probe
atgtgactggcacgggagttgatcctggttttcactaaccactgccactccccaccctctagggttgtcaatgaa

SEQ ID NO: 168 - DNA, 75 bp, Artificial Sequence
  Probe
atgtgactggcacgggagttgatcctggttttcacgagctctaccaatgtgagtgaccattatcactcctacatg

SEQ ID NO: 169 - DNA, 75 bp, Artificial Sequence
  Probe
atgtgactggcacgggagttgatcctggttttcacaaaattgtgattcagtgggtagattctgtgtgtaaagccc

SEQ ID NO: 170 - DNA, 75 bp, Artificial Sequence
  Probe
atgtgactggcacgggagttgatcctggttttcactatgtgctcagttccctcctctatgcaatggaccgaccgt

SEQ ID NO: 171 - DNA, 75 bp, Artificial Sequence
  Probe
atgtgactggcacgggagttgatcctggttttcacgtgtaaattgccgagcacgtagtaaccatgcaacaagtgt

SEQ ID NO: 172 - DNA, 75 bp, Artificial Sequence
  Probe
atgtgactggcacgggagttgatcctggttttcactggggacacagtgtgtgctgccatctcccttctaccggca

SEQ ID NO: 173 - DNA, 75 bp, Artificial Sequence
  Probe
atgtgactggcacgggagttgatcctggttttcacaagagcctttccctctgcccttttcaagcctctgcccatc

SEQ ID NO: 174 - DNA, 75 bp, Artificial Sequence
  Probe
atgtgactggcacgggagttgatcctggttttcacgaccacactgagttctctgtgacctgcaggtcagctcacc

SEQ ID NO: 175 - DNA, 75 bp, Artificial Sequence
  Probe
atgtgactggcacgggagttgatcctggttttcactttcctatctctctgcctggagggtggtggagggctggtt

SEQ ID NO: 176 - DNA, 75 bp, Artificial Sequence
  Probe
atgtgactggcacgggagttgatcctggttttcacaaacaggagctgcgccggtggaagcatgtgggagctagaa

SEQ ID NO: 177 - DNA, 75 bp, Artificial Sequence
  Probe
atgtgactggcacgggagttgatcctggttttcacggacactgaaggagctccccaccccctgatcagccaggag

SEQ ID NO: 178 - DNA, 75 bp, Artificial Sequence
  Probe
atgtgactggcacgggagttgatcctggttttcacgggaactgcagctgctctggtggggggaaggttgggagct

SEQ ID NO: 179 - DNA, 75 bp, Artificial Sequence
  Probe
atgtgactggcacgggagttgatcctggttttcacacccaattccagggactagcataacgaagtgacaccttgg

SEQ ID NO: 180 - DNA, 75 bp, Artificial Sequence
  Probe
atgtgactggcacgggagttgatcctggttttcaccctgcccccttgggagtccctggggctctgtgcactcacc

SEQ ID NO: 181 - DNA, 75 bp, Artificial Sequence
  Probe
atgtgactggcacgggagttgatcctggttttcacggaagcacccccggtattaaaacgaacggggcggaaagaa

SEQ ID NO: 182 - DNA, 75 bp, Artificial Sequence
  Probe
atgtgactggcacgggagttgatcctggttttcacctaacaaaggggacgcgacccggggtccagtgccccaggg

SEQ ID NO: 183 - DNA, 75 bp, Artificial Sequence
  Probe
atgtgactggcacgggagttgatcctggttttcaccctggggggactgggtggcctcacccccaacccggtcatc

SEQ ID NO: 184 - DNA, 75 bp, Artificial Sequence
  Probe
atgtgactggcacgggagttgatcctggttttcaccgcgctccagcttctcgcgggcggagaagccgctccacat

SEQ ID NO: 185 - DNA, 75 bp, Artificial Sequence
  Probe
atgtgactggcacgggagttgatcctggttttcaccccacccggccgccgagtgcgtggatcccgccgtggtctt

SEQ ID NO: 186 - DNA, 75 bp, Artificial Sequence
  Probe
atgtgactggcacgggagttgatcctggttttcacgggcacgggcgctggctcgcgcttgttcacgggaaagggg

SEQ ID NO: 187 - DNA, 75 bp, Artificial Sequence
  Probe
atgtgactggcacgggagttgatcctggttttcacaacatggatatatatgtgaatttcattcaaatggttctca

SEQ ID NO: 188 - DNA, 75 bp, Artificial Sequence
  Probe
atgtgactggcacgggagttgatcctggttttcactaaaccaacattcttaatgtcaacacaatgtttgtttaaa

SEQ ID NO: 189 - DNA, 75 bp, Artificial Sequence
  Probe
atgtgactggcacgggagttgatcctggttttcacccctacgtggagagtgaggatgcacccccacagaagaaga

SEQ ID NO: 190 - DNA, 75 bp, Artificial Sequence
  Probe
atgtgactggcacgggagttgatcctggttttcacatgacactcttgagcggacgtggggacgcctcgctcttta

SEQ ID NO: 191 - DNA, 75 bp, Artificial Sequence
  Probe
atgtgactggcacgggagttgatcctggttttcactctcacgctcagggaccacgtgccggagttggtaaagaat

SEQ ID NO: 192 - DNA, 75 bp, Artificial Sequence
  Probe
atgtgactggcacgggagttgatcctggttttcaccagtggcctttttcaaaatgaccaccttggcggccttctc

SEQ ID NO: 193 - DNA, 75 bp, Artificial Sequence
  Probe
atgtgactggcacgggagttgatcctggttttcacgctagggggctggggttggggtgggggtggtgggcctgcc

SEQ ID NO: 194 - DNA, 75 bp, Artificial Sequence
  Probe
atgtgactggcacgggagttgatcctggttttcaccagtttccataggtctgaaaatgtttcctgactcagaggg

SEQ ID NO: 195 - DNA, 75 bp, Artificial Sequence
  Probe
atgtgactggcacgggagttgatcctggttttcacctgccatggaggagccgcagtcagatcctagcgtcgagcc

SEQ ID NO: 196 - DNA, 75 bp, Artificial Sequence
  Probe
atgtgactggcacgggagttgatcctggttttcactcatgctggatccccacttttcctcttgcagcagccagac

SEQ ID NO: 197 - DNA, 75 bp, Artificial Sequence
  Probe
atgtgactggcacgggagttgatcctggttttcacagccccccagccctccaggtccccagccctccaggtcccc

SEQ ID NO: 198 - DNA, 75 bp, Artificial Sequence
  Probe
atgtgactggcacgggagttgatcctggttttcacgcagagacctgtgggaagcgaaaattccatgggactgact

SEQ ID NO: 199 - DNA, 75 bp, Artificial Sequence
  Probe
atgtgactggcacgggagttgatcctggttttcacgcagggggatacggccaggcattgaagtctcatggaagcc

SEQ ID NO: 200 - DNA, 75 bp, Artificial Sequence
  Probe
atgtgactggcacgggagttgatcctggttttcacccgtgcaagtcacagacttggctgtcccagaatgcaagaa

SEQ ID NO: 201 - DNA, 75 bp, Artificial Sequence
  Probe
atgtgactggcacgggagttgatcctggttttcacccagaaaacctaccagggcagctacggtttccgtctgggc

SEQ ID NO: 202 - DNA, 75 bp, Artificial Sequence
  Probe
atgtgactggcacgggagttgatcctggttttcacgaagggacagaagatgacaggggccaggagggggctggtg

SEQ ID NO: 203 - DNA, 75 bp, Artificial Sequence
  Probe
atgtgactggcacgggagttgatcctggttttcacgtggcccctgcaccagcagctcctacaccggcggcccctg

SEQ ID NO: 204 - DNA, 75 bp, Artificial Sequence
  Probe
atgtgactggcacgggagttgatcctggttttcacggggggagcagcctctggcattctgggagcttcatctgga

SEQ ID NO: 205 - DNA, 75 bp, Artificial Sequence
  Probe
atgtgactggcacgggagttgatcctggttttcacccccggacgatattgaacaatggttcactgaagacccagg

SEQ ID NO: 206 - DNA, 75 bp, Artificial Sequence
  Probe
atgtgactggcacgggagttgatcctggttttcacctggggggctggggggctgaggacctggtcctctgactgc

SEQ ID NO: 207 - DNA, 75 bp, Artificial Sequence
  Probe
atgtgactggcacgggagttgatcctggttttcaccctgggcaaccagccctgtcgtctctccagccccagctgc

SEQ ID NO: 208 - DNA, 75 bp, Artificial Sequence
  Probe
atgtgactggcacgggagttgatcctggttttcacccatcgctatctgagcagcgctcatggtgggggcagcgcc

SEQ ID NO: 209 - DNA, 75 bp, Artificial Sequence
  Probe
atgtgactggcacgggagttgatcctggttttcacgccatctacaagcagtcacagcacatgacggaggttgtga

SEQ ID NO: 210 - DNA, 75 bp, Artificial Sequence
  Probe
atgtgactggcacgggagttgatcctggttttcaccatggcgcggacgcgggtgccgggcgggggtgtggaatca

SEQ ID NO: 211 - DNA, 75 bp, Artificial Sequence
  Probe
atgtgactggcacgggagttgatcctggttttcactttgccaactggccaagacctgccctgtgcagctgtgggt

SEQ ID NO: 212 - DNA, 75 bp, Artificial Sequence
  Probe
atgtgactggcacgggagttgatcctggttttcactgctttatctgttcacttgtgccctgactttcaactctgt

SEQ ID NO: 213 - DNA, 75 bp, Artificial Sequence
  Probe
atgtgactggcacgggagttgatcctggttttcacgagggccactgacaaccacccttaacccctcctcccagag

SEQ ID NO: 214 - DNA, 75 bp, Artificial Sequence
  Probe
atgtgactggcacgggagttgatcctggttttcaccctcaggcggctcatagggcaccaccacactatgtcgaaa

SEQ ID NO: 215 - DNA, 75 bp, Artificial Sequence
  Probe
atgtgactggcacgggagttgatcctggttttcacaggaaatttgcgtgtggagtatttggatgacagaaacact

SEQ ID NO: 216 - DNA, 75 bp, Artificial Sequence
  Probe
atgtgactggcacgggagttgatcctggttttcacccagggtccccaggcctctgattcctcactgattgctctt

SEQ ID NO: 217 - DNA, 75 bp, Artificial Sequence
  Probe
atgtgactggcacgggagttgatcctggttttcacgaggcaagcagaggctggggcacagcaggccagtgtgcag

SEQ ID NO: 218 - DNA, 75 bp, Artificial Sequence
  Probe
atgtgactggcacgggagttgatcctggttttcaccctggagtcttccagtgtgatgatggtgaggatgggcctc

SEQ ID NO: 219 - DNA, 75 bp, Artificial Sequence
  Probe
atgtgactggcacgggagttgatcctggttttcacactacatgtgtaacagttcctgcatgggcggcatgaaccg

SEQ ID NO: 220 - DNA, 75 bp, Artificial Sequence
  Probe
atgtgactggcacgggagttgatcctggttttcaccttgccacaggtctccccaaggcgcactggcctcatcttg

SEQ ID NO: 221 - DNA, 75 bp, Artificial Sequence
  Probe
atgtgactggcacgggagttgatcctggttttcacctgcacccttggtctcctccaccgcttcttgtcctgcttg

SEQ ID NO: 222 - DNA, 75 bp, Artificial Sequence
  Probe
atgtgactggcacgggagttgatcctggttttcaccctcgcttagtgctccctgggggcagctcgtggtgaggct

SEQ ID NO: 223 - DNA, 75 bp, Artificial Sequence
  Probe
atgtgactggcacgggagttgatcctggttttcacgaccggcgcacagaggaagagaatctccgcaagaaagggg

SEQ ID NO: 224 - DNA, 75 bp, Artificial Sequence
  Probe
atgtgactggcacgggagttgatcctggttttcactctcccaggacaggcacaaacacgcacctcaaagctgttc

SEQ ID NO: 225 - DNA, 75 bp, Artificial Sequence
  Probe
atgtgactggcacgggagttgatcctggttttcactctcttttcctatcctgagtagtggtaatctactgggacg

SEQ ID NO: 226 - DNA, 75 bp, Artificial Sequence
  Probe
atgtgactggcacgggagttgatcctggttttcacggacaggtaggacctgatttccttactgcctcttgcttct

SEQ ID NO: 227 - DNA, 75 bp, Artificial Sequence
  Probe
atgtgactggcacgggagttgatcctggttttcacggcattttgagtgttagactggaaactttccacttgataa

SEQ ID NO: 228 - DNA, 75 bp, Artificial Sequence
  Probe
atgtgactggcacgggagttgatcctggttttcaccctgaagggtgaaatattctccatccagtggtttcttctt

SEQ ID NO: 229 - DNA, 75 bp, Artificial Sequence
  Probe
atgtgactggcacgggagttgatcctggttttcaccctagcactgcccaacaacaccagctcctctccccagcca

SEQ ID NO: 230 - DNA, 75 bp, Artificial Sequence
  Probe
atgtgactggcacgggagttgatcctggttttcactgcctcagattcacttttatcacctttccttgcctctttc

SEQ ID NO: 231 - DNA, 75 bp, Artificial Sequence
  Probe
atgtgactggcacgggagttgatcctggttttcacatggctttccaacctaggaaggcaggggagtagggccagg

SEQ ID NO: 232 - DNA, 75 bp, Artificial Sequence
  Probe
atgtgactggcacgggagttgatcctggttttcaccctggagtgagccctgctcccccctggctccttcccagcc

SEQ ID NO: 233 - DNA, 75 bp, Artificial Sequence
  Probe
atgtgactggcacgggagttgatcctggttttcactccgagagctgaatgaggccttggaactcaaggatgccca

SEQ ID NO: 234 - DNA, 75 bp, Artificial Sequence
  Probe
atgtgactggcacgggagttgatcctggttttcaccatcttttaactcaggtactgtgtatatacttacttctcc

SEQ ID NO: 235 - DNA, 75 bp, Artificial Sequence
  Probe
atgtgactggcacgggagttgatcctggttttcacggcaggggagggagagatgggggtgggaggctgtcagtgg

SEQ ID NO: 236 - DNA, 75 bp, Artificial Sequence
  Probe
atgtgactggcacgggagttgatcctggttttcacgtcagtctgagtcaggcccttctgtcttgaacatgagttt

SEQ ID NO: 237 - DNA, 75 bp, Artificial Sequence
  Probe
atgtgactggcacgggagttgatcctggttttcaccctgaagtccaaaaagggtcagtctacctcccgccataaa

SEQ ID NO: 238 - DNA, 75 bp, Artificial Sequence
  Probe
atgtgactggcacgggagttgatcctggttttcacggcacagaccctctcactcatgtgatgtcatctctcctcc

SEQ ID NO: 239 - DNA, 75 bp, Artificial Sequence
  Probe
atgtgactggcacgggagttgatcctggttttcaccaggggcttatgtgtctccttgatgacctgcggcgacgtc

SEQ ID NO: 240 - DNA, 75 bp, Artificial Sequence
  Probe
atgtgactggcacgggagttgatcctggttttcacccatcatctcctcccttccccttctgcccaggctgttgca

SEQ ID NO: 241 - DNA, 75 bp, Artificial Sequence
  Probe
atgtgactggcacgggagttgatcctggttttcacaattctggcttctccctgctcacactttcttccattgcat

SEQ ID NO: 242 - DNA, 75 bp, Artificial Sequence
  Probe
atgtgactggcacgggagttgatcctggttttcacgtcagctcgtgttggcaacataccatcttcaacctctgca

SEQ ID NO: 243 - DNA, 75 bp, Artificial Sequence
  Probe
atgtgactggcacgggagttgatcctggttttcactaatttcttggcccctcttcggtaaccctgagccaaatgt

SEQ ID NO: 244 - DNA, 75 bp, Artificial Sequence
  Probe
atgtgactggcacgggagttgatcctggttttcacggtgaaataaaggaagatactagttttgctgaaaatgaca

SEQ ID NO: 245 - DNA, 75 bp, Artificial Sequence
  Probe
atgtgactggcacgggagttgatcctggttttcacactcatttgtatctgaagtggaaccaaatgatactgatcc

SEQ ID NO: 246 - DNA, 75 bp, Artificial Sequence
  Probe
atgtgactggcacgggagttgatcctggttttcacagttgagaccattcacaggccaaagacggtacaacttcct

SEQ ID NO: 247 - DNA, 75 bp, Artificial Sequence
  Probe
atgtgactggcacgggagttgatcctggttttcacgaaaatgaatgctctgagctttggaagctctcagggtaca

SEQ ID NO: 248 - DNA, 75 bp, Artificial Sequence
  Probe
atgtgactggcacgggagttgatcctggttttcacgggccatcgcgatgtcgcacggtacctgcgcgcggctgcg

SEQ ID NO: 249 - DNA, 75 bp, Artificial Sequence
  Probe
atgtgactggcacgggagttgatcctggttttcacccccatccagcttcaaaagctcttcgaatcattgatgtgc

SEQ ID NO: 250 - DNA, 75 bp, Artificial Sequence
  Probe
atgtgactggcacgggagttgatcctggttttcactgccaagcctgaactacccctcttttacactcctattgat

SEQ ID NO: 251 - DNA, 75 bp, Artificial Sequence
  Probe
atgtgactggcacgggagttgatcctggttttcacccaccctgactgtgctctgtccccccagggctggacatcc

SEQ ID NO: 252 - DNA, 75 bp, Artificial Sequence
  Probe
atgtgactggcacgggagttgatcctggttttcacagtcaggagtgggatgatcttataaaactcgtagaaagag

SEQ ID NO: 253 - DNA, 75 bp, Artificial Sequence
  Probe
atgtgactggcacgggagttgatcctggttttcaccttcggggagacaacgacggcggtggcgggagcttctcca

SEQ ID NO: 254 - DNA, 75 bp, Artificial Sequence
  Probe
atgtgactggcacgggagttgatcctggttttcaccatacagtcctggatgatgatgtttttgatgaaggtctcg

SEQ ID NO: 255 - DNA, 75 bp, Artificial Sequence
  Probe
atgtgactggcacgggagttgatcctggttttcacttttactgttcttcctcagacattcaaacgtgttttgatc

SEQ ID NO: 256 - DNA, 75 bp, Artificial Sequence
  Probe
atgtgactggcacgggagttgatcctggttttcacgtggaagcatactgcaaaatatttgttttcagtctctgca

SEQ ID NO: 257 - DNA, 75 bp, Artificial Sequence
  Probe
atgtgactggcacgggagttgatcctggttttcacacgtacccctctcagcccctcctcttggactccagccatg

SEQ ID NO: 258 - DNA, 75 bp, Artificial Sequence
  Probe
atgtgactggcacgggagttgatcctggttttcacgtggcgtaagcgcggcacgcggcgcagtggtccccgtcct

SEQ ID NO: 259 - DNA, 21 bp, Artificial Sequence
  Adaptor
  misc_feature (1)..(5): n is a, c, g, or t
nnnnnaagatcttagtggcac

SEQ ID NO: 260 - DNA, 21 bp, Artificial Sequence
  Adaptor
  misc_feature (1)..(5): n is a, c, g, or t
nnnnncgacagaactattgcc

SEQ ID NO: 261 - DNA, 21 bp, Artificial Sequence
  Adaptor
  misc_feature: n is a, c, g, or t
  misc_feature (1)..(5): n is a, c, g, or t
nnnnnactatcttagtggcac

SEQ ID NO: 262 - DNA, 21 bp, Artificial Sequence
  Adaptor
  misc_feature (1)..(5): n is a, c, g, or t
nnnnnctccagaactattgcc

SEQ ID NO: 263 - DNA, 21 bp, Artificial Sequence
  Adaptor
  misc_feature (1)..(5): n is a, c, g, or t
nnnnnagcatcttagtggcac

SEQ ID NO: 264 - DNA, 21 bp, Artificial Sequence
  Adaptor
  misc_feature (1)..(5): n is a, c, g, or t
nnnnncatcagaactattgcc

SEQ ID NO: 265 - DNA, 21 bp, Artificial Sequence
  Adaptor
  misc_feature (1)..(5): n is a, c, g, or t
nnnnnataatcttagtggcac

SEQ ID NO: 266 - DNA, 21 bp, Artificial Sequence
  Adaptor
  misc_feature (1)..(5): n is a, c, g, or t
nnnnnaagaaggtagaccctc

SEQ ID NO: 267 - DNA, 21 bp, Artificial Sequence
  Adaptor
  misc_feature (1)..(5): n is a, c, g, or t
nnnnntttctctactcgtgac

SEQ ID NO: 268 - DNA, 21 bp, Artificial Sequence
  Adaptor
  misc_feature (1)..(5): n is a, c, g, or t
nnnnnactaaggtagaccctc

SEQ ID NO: 269 - DNA, 21 bp, Artificial Sequence
  Adaptor
  misc_feature (1)..(5): n is a, c, g, or t
nnnnngaagctacgagtatcc

SEQ ID NO: 270 - DNA, 21 bp, Artificial Sequence
  Adaptor
  misc_feature (1)..(5): n is a, c, g, or t
nnnnnagcaaggtagaccctc

SEQ ID NO: 271 - DNA, 21 bp, Artificial Sequence
  Adaptor
  misc_feature (1)..(5): n is a, c, g, or t
nnnnncattgacgtctagagc

SEQ ID NO: 272 - DNA, 21 bp, Artificial Sequence
  Adaptor
  misc_feature (1)..(5): n is a, c, g, or t
nnnnntcactctactcgtgac

SEQ ID NO: 273 - DNA, 21 bp, Artificial Sequence
  Adaptor
  misc_feature (1)..(5): n is a, c, g, or t
nnnnnataaaggtagaccctc

SEQ ID NO: 274 - DNA, 21 bp, Artificial Sequence
  Adaptor
  misc_feature (1)..(5): n is a, c, g, or t
nnnnntacctctactcgtgac

SEQ ID NO: 275 - DNA, 20 bp, Artificial Sequence
  Adaptor
  misc_feature (1)..(5): n is a, c, g, or t
nnnnnttttgtgtgtgtgtg

SEQ ID NO: 276 - DNA, 20 bp, Artificial Sequence
  Adaptor
  misc_feature (1)..(5): n is a, c, g, or t
nnnnnactacacacacacac

SEQ ID NO: 277 - DNA, 20 bp, Artificial Sequence
  Adaptor
  misc_feature (1)..(5): n is a, c, g, or t
nnnnnctcgtgtgtgtgtgt

SEQ ID NO: 278 - DNA, 20 bp, Artificial Sequence
  Adaptor
  misc_feature (1)..(5): n is a, c, g, or t
nnnnngaacacacacacaca

SEQ ID NO: 279 - DNA, 20 bp, Artificial Sequence
  Adaptor
  misc_feature (1)..(5): n is a, c, g, or t
nnnnncatgtgtgtgtgtgt

SEQ ID NO: 280 - DNA, 20 bp, Artificial Sequence
  Adaptor
  misc_feature (1)..(5): n is a, c, g, or t
nnnnngtgcacacacacaca

SEQ ID NO: 281 - DNA, 20 bp, Artificial Sequence
  Adaptor
  misc_feature (1)..(5): n is a, c, g, or t
nnnnnataacacacacacac

SEQ ID NO: 282 - DNA, 20 bp, Artificial Sequence
  Adaptor
  misc_feature (1)..(5): n is a, c, g, or t
nnnnntactgtgtgtgtgtg

SEQ ID NO: 283 - DNA, 25 bp, Artificial Sequence
  Primer
tgcaggaccagagaattcgaataca

SEQ ID NO: 284 - DNA, 58 bp, Artificial Sequence; identical to SEQ ID NO: 152
  Primer

SEQ ID NO: 285 - DNA, 18 bp, Artificial Sequence
  Primer
cggtggctcacgcctgta

SEQ ID NO: 286 - DNA, 18 bp, Artificial Sequence
  Primer
gcctcggcctcccaaagt

SEQ ID NO: 287 - DNA, 21 bp, Artificial Sequence
  Primer
gaggctgaggcaggagaatcg

SEQ ID NO: 288 - DNA, 18 bp, Artificial Sequence
  Primer
gtcgcccaggctggagtg

SEQ ID NO: 289 - DNA, 25 bp, Artificial Sequence
  Element 1
tgcaggaccagagaattcgaataca

SEQ ID NO: 290 - DNA, 5 bp, Artificial Sequence
  Element 2
cgggt

SEQ ID NO: 291 - DNA, 5 bp, Artificial Sequence
  Element 2
cggtg

SEQ ID NO: 292 - DNA, 5 bp, Artificial Sequence
  Element 2
cgtgg

SEQ ID NO: 293 - DNA, 5 bp, Artificial Sequence
  Element 2
gcggt

SEQ ID NO: 294 - DNA, 5 bp, Artificial Sequence
  Element 2
gcgtg

SEQ ID NO: 295 - DNA, 5 bp, Artificial Sequence
  Element 2
gctgg

SEQ ID NO: 296 - DNA, 5 bp, Artificial Sequence
  Element 2
ggcgt

SEQ ID NO: 297 - DNA, 5 bp, Artificial Sequence
  Element 2
ggctg

SEQ ID NO: 298 - DNA, 5 bp, Artificial Sequence
  Element 2
gggct

SEQ ID NO: 299 - DNA, 5 bp, Artificial Sequence
  Element 2
ttaaa

SEQ ID NO: 300 - DNA, 5 bp, Artificial Sequence
  Element 2
ttacc

SEQ ID NO: 301 - DNA, 5 bp, Artificial Sequence
  Element 2
ttatt

SEQ ID NO: 302 - DNA, 5 bp, Artificial Sequence
  Element 2
ttcac

SEQ ID NO: 303 - DNA, 5 bp, Artificial Sequence
  Element 2
ttcca

SEQ ID NO: 304 - DNA, 5 bp, Artificial Sequence
  Element 2
tttat

SEQ ID NO: 305 - DNA, 5 bp, Artificial Sequence
  Element 2
tttta

SEQ ID NO: 306 - DNA, 5 bp, Artificial Sequence
  Element 2
gcacg

SEQ ID NO: 307 - DNA, 5 bp, Artificial Sequence
  Element 2
gcagc

SEQ ID NO: 308 - DNA, 5 bp, Artificial Sequence
  Element 2
gccag

SEQ ID NO: 309 - DNA, 5 bp, Artificial Sequence
  Element 2
gccga

SEQ ID NO: 310 - DNA, 5 bp, Artificial Sequence
  Element 2
gcgac

SEQ ID NO: 311 - DNA, 5 bp, Artificial Sequence
  Element 2
gcgca

SEQ ID NO: 312 - DNA, 5 bp, Artificial Sequence
  Element 2
ggaaa

SEQ ID NO: 313 - DNA, 5 bp, Artificial Sequence
  Element 2
ggacc

SEQ ID NO: 314 - DNA, 5 bp, Artificial Sequence
  Element 2
ggatt

SEQ ID NO: 315 - DNA, 5 bp, Artificial Sequence
  Element 2
ggcac

SEQ ID NO: 316 - DNA, 5 bp, Artificial Sequence
  Element 2
ggcca

SEQ ID NO: 317 - DNA, 5 bp, Artificial Sequence
  Element 2
ggtat

SEQ ID NO: 318 - DNA, 5 bp, Artificial Sequence
  Element 2
ggtta

SEQ ID NO: 319 - DNA, 5 bp, Artificial Sequence
  Element 2
gtagt

SEQ ID NO: 320 - DNA, 5 bp, Artificial Sequence
  Element 2
gtatg

SEQ ID NO: 321 - DNA, 5 bp, Artificial Sequence
  Element 2
gtgat

SEQ ID NO: 322 - DNA, 5 bp, Artificial Sequence
  Element 2
ccgtc

SEQ ID NO: 323 - DNA, 5 bp, Artificial Sequence
  Element 2
cctcg

SEQ ID NO: 324 - DNA, 5 bp, Artificial Sequence
  Element 2
cctgc

SEQ ID NO: 325 - DNA, 5 bp, Artificial Sequence
  Element 2
cgaat

SEQ ID NO: 326 - DNA, 5 bp, Artificial Sequence
  Element 2
cgata

SEQ ID NO: 327 - DNA, 5 bp, Artificial Sequence
  Element 2
cgcct

SEQ ID NO: 328 - DNA, 5 bp, Artificial Sequence
  Element 2
cgctc

SEQ ID NO: 329 - DNA, 5 bp, Artificial Sequence
  Element 2
cgtaa

SEQ ID NO: 330 - DNA, 5 bp, Artificial Sequence
  Element 2
cgtcc

SEQ ID NO: 331 - DNA, 5 bp, Artificial Sequence
  Element 2
cgttt

SEQ ID NO: 332 - DNA, 5 bp, Artificial Sequence
  Element 2
ctaag

SEQ ID NO: 333 - DNA, 5 bp, Artificial Sequence
  Element 2
ctaga

SEQ ID NO: 334 - DNA, 5 bp, Artificial Sequence
  Element 2
ctccg

SEQ ID NO: 335 - DNA, 5 bp, Artificial Sequence
  Element 2
ctcgc

SEQ ID NO: 336 - DNA, 5 bp, Artificial Sequence
  Element 2
ctgaa

SEQ ID NO: 337 - DNA, 5 bp, Artificial Sequence
  Element 2
ctgcc

SEQ ID NO: 338 - DNA, 5 bp, Artificial Sequence
  Element 2
ttgtc

SEQ ID NO: 339 - DNA, 5 bp, Artificial Sequence
  Element 2
tttcg

SEQ ID NO: 340 - DNA, 5 bp, Artificial Sequence
  Element 2
tttgc

SEQ ID NO: 341 - DNA, 5 bp, Artificial Sequence
  Element 2
aaaaa

SEQ ID NO: 342 - DNA, 5 bp, Artificial Sequence
  Element 2
aaacc

SEQ ID NO: 343 - DNA, 5 bp, Artificial Sequence
  Element 2
aaatt

SEQ ID NO: 344 - DNA, 5 bp, Artificial Sequence
  Element 2
aacac

SEQ ID NO: 345 - DNA, 5 bp, Artificial Sequence
  Element 2
aacca

SEQ ID NO: 346 - DNA, 5 bp, Artificial Sequence
  Element 2
aatat

SEQ ID NO: 347 - DNA, 5 bp, Artificial Sequence
  Element 2
aatta

SEQ ID NO: 348 - DNA, 5 bp, Artificial Sequence
  Element 2
acaac

SEQ ID NO: 349 - DNA, 5 bp, Artificial Sequence
  Element 2
acaca

SEQ ID NO: 350 - DNA, 5 bp, Artificial Sequence
  Element 2
accaa

SEQ ID NO: 351 - DNA, 5 bp, Artificial Sequence
  Element 2
acccc

SEQ ID NO: 352 - DNA, 5 bp, Artificial Sequence
  Element 2
acctt

SEQ ID NO: 353 - DNA, 5 bp, Artificial Sequence
  Element 2
actct

SEQ ID NO: 354 - DNA, 5 bp, Artificial Sequence
  Element 2
gggtc

SEQ ID NO: 355 - DNA, 5 bp, Artificial Sequence
  Element 2
ggtcg

SEQ ID NO: 356 - DNA, 5 bp, Artificial Sequence
  Element 2
ggtgc

SEQ ID NO: 357 - DNA, 5 bp, Artificial Sequence
  Element 2
gtcgg

SEQ ID NO: 358 - DNA, 5 bp, Artificial Sequence
  Element 2
gtgcg

SEQ ID NO: 359 - DNA, 5 bp, Artificial Sequence
  Element 2
gtggc

SEQ ID NO: 360 - DNA, 5 bp, Artificial Sequence
  Element 2
tgcgg

SEQ ID NO: 361 - DNA, 5 bp, Artificial Sequence
  Element 2
tggcg

SEQ ID NO: 362 - DNA, 5 bp, Artificial Sequence
  Element 2
tgggc

SEQ ID NO: 363 - DNA, 5 bp, Artificial Sequence
  Element 2
aaagg

SEQ ID NO: 364 - DNA, 5 bp, Artificial Sequence
  Element 2
aagag

SEQ ID NO: 365 - DNA, 5 bp, Artificial Sequence
  Element 2
aagga

SEQ ID NO: 366 - DNA, 5 bp, Artificial Sequence
  Element 2
accgg

SEQ ID NO: 367 - DNA, 5 bp, Artificial Sequence
  Element 2
acgcg

SEQ ID NO: 368 - DNA, 5 bp, Artificial Sequence
  Element 2
acggc

SEQ ID NO: 369 - DNA, 5 bp, Artificial Sequence
  Element 2
agaag

SEQ ID NO: 370 - DNA, 5 bp, Artificial Sequence
  Element 2
gtgta

SEQ ID NO: 371 - DNA, 5 bp, Artificial Sequence
  Element 2
gttag

SEQ ID NO: 372 - DNA, 5 bp, Artificial Sequence
  Element 2
gttga

SEQ ID NO: 373 - DNA, 5 bp, Artificial Sequence
  Element 2
taggt

SEQ ID NO: 374 - DNA, 5 bp, Artificial Sequence
  Element 2
tagtg

SEQ ID NO: 375 - DNA, 5 bp, Artificial Sequence
  Element 2
tatgg

SEQ ID NO: 376 - DNA, 5 bp, Artificial Sequence
  Element 2
tgagt

SEQ ID NO: 377 - DNA, 5 bp, Artificial Sequence
  Element 2
tgatg

SEQ ID NO: 378 - DNA, 5 bp, Artificial Sequence
  Element 2
tggat

SEQ ID NO: 379 - DNA, 5 bp, Artificial Sequence
  Element 2
tggta

SEQ ID NO: 380 - DNA, 5 bp, Artificial Sequence
  Element 2
tgtag

SEQ ID NO: 381 - DNA, 5 bp, Artificial Sequence
  Element 2
tgtga

SEQ ID NO: 382 - DNA, 5 bp, Artificial Sequence
  Element 2
ttagg

SEQ ID NO: 383 - DNA, 5 bp, Artificial Sequence
  Element 2
ttgag

SEQ ID NO: 384 - DNA, 5 bp, Artificial Sequence
  Element 2
ttgga

SEQ ID NO: 385 - DNA, 5 bp, Artificial Sequence
  Element 2
aacgt

SEQ ID NO: 386 - DNA, 5 bp, Artificial Sequence
  Element 2
ctgtt

SEQ ID NO: 387 - DNA, 5 bp, Artificial Sequence
  Element 2
cttgt

SEQ ID NO: 388 - DNA, 5 bp, Artificial Sequence
  Element 2
ctttg

SEQ ID NO: 389 - DNA, 5 bp, Artificial Sequence
  Element 2
gaact

SEQ ID NO: 390 - DNA, 5 bp, Artificial Sequence
  Element 2
gaatc

SEQ ID NO: 391 - DNA, 5 bp, Artificial Sequence
  Element 2
gacat

SEQ ID NO: 392 - DNA, 5 bp, Artificial Sequence
  Element 2
gacta

SEQ ID NO: 393 - DNA, 5 bp, Artificial Sequence
  Element 2
gatac

SEQ ID NO: 394 - DNA, 5 bp, Artificial Sequence
  Element 2
gatca

SEQ ID NO: 395 - DNA, 5 bp, Artificial Sequence
  Element 2
gcaat

SEQ ID NO: 396 - DNA, 5 bp, Artificial Sequence
  Element 2
gcata

SEQ ID NO: 397 - DNA, 5 bp, Artificial Sequence
  Element 2
gccct

SEQ ID NO: 398 - DNA, 5 bp, Artificial Sequence
  Element 2
gcctc

SEQ ID NO: 399 - DNA, 5 bp, Artificial Sequence
  Element 2
gctaa

SEQ ID NO: 400 - DNA, 5 bp, Artificial Sequence
  Element 2
gctcc

SEQ ID NO: 401 - DNA, 5 bp, Artificial Sequence
  Element 2
gcttt

SEQ ID NO: 402 - DNA, 5 bp, Artificial Sequence
  Element 2
acttc

SEQ ID NO: 403 - DNA, 5 bp, Artificial Sequence
  Element 2
ataat

SEQ ID NO: 404 - DNA, 5 bp, Artificial Sequence
  Element 2
atata

SEQ ID NO: 405 - DNA, 5 bp, Artificial Sequence
  Element 2
atcct

SEQ ID NO: 406 - DNA, 5 bp, Artificial Sequence
  Element 2
atctc

SEQ ID NO: 407 - DNA, 5 bp, Artificial Sequence
  Element 2
attaa

SEQ ID NO: 408 - DNA, 5 bp, Artificial Sequence
  Element 2
attcc

SEQ ID NO: 409 - DNA, 5 bp, Artificial Sequence
  Element 2
atttt

SEQ ID NO: 410 - DNA, 5 bp, Artificial Sequence
  Element 2
caaac

SEQ ID NO: 411 - DNA, 5 bp, Artificial Sequence
  Element 2
caaca

SEQ ID NO: 412 - DNA, 5 bp, Artificial Sequence
  Element 2
cacaa

SEQ ID NO: 413 - DNA, 5 bp, Artificial Sequence
  Element 2
caccc

SEQ ID NO: 414 - DNA, 5 bp, Artificial Sequence
  Element 2
cactt

SEQ ID NO: 415 - DNA, 5 bp, Artificial Sequence
  Element 2
catct

SEQ ID NO: 416 - DNA, 5 bp, Artificial Sequence
  Element 2
cattc

SEQ ID NO: 417 - DNA, 5 bp, Artificial Sequence
  Element 2
ccaaa

SEQ ID NO: 418 - DNA, 5 bp, Artificial Sequence
  Element 2
agaga

SEQ ID NO: 419 - DNA, 5 bp, Artificial Sequence
  Element 2
agccg

SEQ ID NO: 420 - DNA, 5 bp, Artificial Sequence
  Element 2
agcgc

SEQ ID NO: 421 - DNA, 5 bp, Artificial Sequence
  Element 2
aggaa

SEQ ID NO: 422 - DNA, 5 bp, Artificial Sequence
  Element 2
aggcc

SEQ ID NO: 423 - DNA, 5 bp, Artificial Sequence
  Element 2
aggtt

SEQ ID NO: 424 - DNA, 5 bp, Artificial Sequence
  Element 2
agtgt

SEQ ID NO: 425 - DNA, 5 bp, Artificial Sequence
  Element 2
agttg

SEQ ID NO: 426 - DNA, 5 bp, Artificial Sequence
  Element 2
atggt

SEQ ID NO: 427 - DNA, 5 bp, Artificial Sequence
  Element 2
atgtg

SEQ ID NO: 428 - DNA, 5 bp, Artificial Sequence
  Element 2
attgg

SEQ ID NO: 429 - DNA, 5 bp, Artificial Sequence
  Element 2
cacgg

SEQ ID NO: 430 - DNA, 5 bp, Artificial Sequence
  Element 2
cagcg

SEQ ID NO: 431 - DNA, 5 bp, Artificial Sequence
  Element 2
caggc

SEQ ID NO: 432 - DNA, 5 bp, Artificial Sequence
  Element 2
ccagg

SEQ ID NO: 433 - DNA, 5 bp, Artificial Sequence
  Element 2
ccgag

SEQ ID NO: 434 - DNA, 5 bp, Artificial Sequence
  Element 2
aactg

SEQ ID NO: 435 - DNA, 5 bp, Artificial Sequence
  Element 2
aagct

SEQ ID NO: 436 - DNA, 5 bp, Artificial Sequence
  Element 2
aagtc

SEQ ID NO: 437 - DNA, 5 bp, Artificial Sequence
  Element 2
aatcg

SEQ ID NO: 438 - DNA, 5 bp, Artificial Sequence
  Element 2
aatgc

SEQ ID NO: 439 - DNA, 5 bp, Artificial Sequence
  Element 2
acagt

SEQ ID NO: 440 - DNA, 5 bp, Artificial Sequence
  Element 2
acatg

SEQ ID NO: 441 - DNA, 5 bp, Artificial Sequence
  Element 2
acgat

SEQ ID NO: 442 - DNA, 5 bp, Artificial Sequence
  Element 2
acgta

SEQ ID NO: 443 - DNA, 5 bp, Artificial Sequence
  Element 2
actag

SEQ ID NO: 444 - DNA, 5 bp, Artificial Sequence
  Element 2
actga

SEQ ID NO: 445 - DNA, 5 bp, Artificial Sequence
  Element 2
agact

SEQ ID NO: 446 - DNA, 5 bp, Artificial Sequence
  Element 2
agatc

SEQ ID NO: 447 - DNA, 5 bp, Artificial Sequence
  Element 2
agcat

SEQ ID NO: 448 - DNA, 5 bp, Artificial Sequence
  Element 2
agcta

SEQ ID NO: 449 - DNA, 5 bp, Artificial Sequence
  Element 2
agtac

SEQ ID NO: 450 - DNA, 5 bp, Artificial Sequence
  Element 2
gtaac

SEQ ID NO: 451 - DNA, 5 bp, Artificial Sequence
  Element 2
gtaca

SEQ ID NO: 452 - DNA, 5 bp, Artificial Sequence
  Element 2
gtcaa

SEQ ID NO: 453 - DNA, 5 bp, Artificial Sequence
  Element 2
gtccc

SEQ ID NO: 454 - DNA, 5 bp, Artificial Sequence
  Element 2
gtctt

SEQ ID NO: 455 - DNA, 5 bp, Artificial Sequence
  Element 2
gttct

SEQ ID NO: 456 - DNA, 5 bp, Artificial Sequence
  Element 2
gtttc

SEQ ID NO: 457 - DNA, 5 bp, Artificial Sequence
  Element 2
taacg

SEQ ID NO: 458 - DNA, 5 bp, Artificial Sequence
  Element 2
taagc

SEQ ID NO: 459 - DNA, 5 bp, Artificial Sequence
  Element 2
tacag

SEQ ID NO: 460 - DNA, 5 bp, Artificial Sequence
  Element 2
tacga

SEQ ID NO: 461 - DNA, 5 bp, Artificial Sequence
  Element 2
tagac

SEQ ID NO: 462 - DNA, 5 bp, Artificial Sequence
  Element 2
tagca

SEQ ID NO: 463 - DNA, 5 bp, Artificial Sequence
  Element 2
tcaag

SEQ ID NO: 464 - DNA, 5 bp, Artificial Sequence
  Element 2
tcaga

SEQ ID NO: 465 - DNA, 5 bp, Artificial Sequence
  Element 2
tcccg

SEQ ID NO: 466 - DNA, 5 bp, Artificial Sequence
  Element 2
ccacc

SEQ ID NO: 467 - DNA, 5 bp, Artificial Sequence
  Element 2
ccatt

SEQ ID NO: 468 - DNA, 5 bp, Artificial Sequence
  Element 2
cccac

SEQ ID NO: 469 - DNA, 5 bp, Artificial Sequence
  Element 2
cccca

SEQ ID NO: 470 - DNA, 5 bp, Artificial Sequence
  Element 2
cctat

SEQ ID NO: 471 - DNA, 5 bp, Artificial Sequence
  Element 2
cctta

SEQ ID NO: 472 - DNA, 5 bp, Artificial Sequence
  Element 2
ctact

SEQ ID NO: 473 - DNA, 5 bp, Artificial Sequence
  Element 2
ctatc

SEQ ID NO: 474 - DNA, 5 bp, Artificial Sequence
  Element 2
ctcat

SEQ ID NO: 475 - DNA, 5 bp, Artificial Sequence
  Element 2
ctcta

SEQ ID NO: 476 - DNA, 5 bp, Artificial Sequence
  Element 2
cttac

SEQ ID NO: 477 - DNA, 5 bp, Artificial Sequence
  Element 2
cttca

SEQ ID NO: 478 - DNA, 5 bp, Artificial Sequence
  Element 2
taaat

SEQ ID NO: 479 - DNA, 5 bp, Artificial Sequence
  Element 2
taata

SEQ ID NO: 480 - DNA, 5 bp, Artificial Sequence
  Element 2
tacct

SEQ ID NO: 481 - DNA, 5 bp, Artificial Sequence
  Element 2
tactc

SEQ ID NO: 482 - DNA, 5 bp, Artificial Sequence
  Element 2
ccgga

SEQ ID NO: 483 - DNA, 5 bp, Artificial Sequence
  Element 2
cgacg

SEQ ID NO: 484 - DNA, 5 bp, Artificial Sequence
  Element 2
cgagc

SEQ ID NO: 485 - DNA, 5 bp, Artificial Sequence
  Element 2
cgcag

SEQ ID NO: 486 - DNA, 5 bp, Artificial Sequence
  Element 2
cgcga

SEQ ID NO: 487 - DNA, 5 bp, Artificial Sequence
  Element 2
cggac

SEQ ID NO: 488 - DNA, 5 bp, Artificial Sequence
  Element 2
cggca

SEQ ID NO: 489 - DNA, 5 bp, Artificial Sequence
  Element 2
gaaag

SEQ ID NO: 490 - DNA, 5 bp, Artificial Sequence
  Element 2
gaaga

SEQ ID NO: 491 - DNA, 5 bp, Artificial Sequence
  Element 2
gaccg

SEQ ID NO: 492 - DNA, 5 bp, Artificial Sequence
  Element 2
gacgc

SEQ ID NO: 493 - DNA, 5 bp, Artificial Sequence
  Element 2
gagaa

SEQ ID NO: 494 - DNA, 5 bp, Artificial Sequence
  Element 2
gagcc

SEQ ID NO: 495 - DNA, 5 bp, Artificial Sequence
  Element 2
gagtt

SEQ ID NO: 496 - DNA, 5 bp, Artificial Sequence
  Element 2
gatgt

SEQ ID NO: 497 - DNA, 5 bp, Artificial Sequence
  Element 2
gattg

SEQ ID NO: 498 - DNA, 5 bp, Artificial Sequence
  Element 2
agtca

SEQ ID NO: 499 - DNA, 5 bp, Artificial Sequence
  Element 2
atacg

SEQ ID NO: 500 - DNA, 5 bp, Artificial Sequence
  Element 2
atagc

SEQ ID NO: 501 - DNA, 5 bp, Artificial Sequence
  Element 2
atcag

SEQ ID NO: 502 - DNA, 5 bp, Artificial Sequence
  Element 2
atcga

SEQ ID NO: 503 - DNA, 5 bp, Artificial Sequence
  Element 2
atgac

SEQ ID NO: 504 - DNA, 5 bp, Artificial Sequence
  Element 2
atgca

SEQ ID NO: 505 - DNA, 5 bp, Artificial Sequence
  Element 2
caagt

SEQ ID NO: 506 - DNA, 5 bp, Artificial Sequence
  Element 2
caatg

SEQ ID NO: 507 - DNA, 5 bp, Artificial Sequence
  Element 2
cagat

SEQ ID NO: 508 - DNA, 5 bp, Artificial Sequence
  Element 2
cagta

SEQ ID NO: 509 - DNA, 5 bp, Artificial Sequence
  Element 2
catag

SEQ ID NO: 510 - DNA, 5 bp, Artificial Sequence
  Element 2
catga

SEQ ID NO: 511 - DNA, 5 bp, Artificial Sequence
  Element 2
cccgt

SEQ ID NO: 512 - DNA, 5 bp, Artificial Sequence
  Element 2
ccctg

SEQ ID NO: 513 - DNA, 5 bp, Artificial Sequence
  Element 2
ccgct

SEQ ID NO: 514 - DNA, 5 bp, Artificial Sequence
  Element 2
tccgc

SEQ ID NO: 515 - DNA, 5 bp, Artificial Sequence
  Element 2
tcgaa

SEQ ID NO: 516 - DNA, 5 bp, Artificial Sequence
  Element 2
tcgcc

SEQ ID NO: 517 - DNA, 5 bp, Artificial Sequence
  Element 2
tcgtt

SEQ ID NO: 518 - DNA, 5 bp, Artificial Sequence
  Element 2
tctgt

SEQ ID NO: 519 - DNA, 5 bp, Artificial Sequence
  Element 2
tcttg

SEQ ID NO: 520 - DNA, 5 bp, Artificial Sequence
  Element 2
tgaac

SEQ ID NO: 521 - DNA, 5 bp, Artificial Sequence
  Element 2
tgaca

SEQ ID NO: 522 - DNA, 5 bp, Artificial Sequence
  Element 2
tgcaa

SEQ ID NO: 523 - DNA, 5 bp, Artificial Sequence
  Element 2
tgccc

SEQ ID NO: 524 - DNA, 5 bp, Artificial Sequence
  Element 2
tgctt

SEQ ID NO: 525 - DNA, 5 bp, Artificial Sequence
  Element 2
tgtct

SEQ ID NO: 526 - DNA, 5 bp, Artificial Sequence
  Element 2
tgttc

SEQ ID NO: 527 - DNA, 5 bp, Artificial Sequence
  Element 2
ttcgt

SEQ ID NO: 528 - DNA, 5 bp, Artificial Sequence
  Element 2
ttctg

SEQ ID NO: 529 - DNA, 5 bp, Artificial Sequence
  Element 2
ttgct

SEQ ID NO: 530 - DNA, 5 bp, Artificial Sequence
  Element 2
tataa

SEQ ID NO: 531 - DNA, 5 bp, Artificial Sequence
  Element 2
tatcc

SEQ ID NO: 532 - DNA, 5 bp, Artificial Sequence
  Element 2
tattt

SEQ ID NO: 533 - DNA, 5 bp, Artificial Sequence
  Element 2
tcact

SEQ ID NO: 534 - DNA, 5 bp, Artificial Sequence
  Element 2
tcatc

SEQ ID NO: 535 - DNA, 5 bp, Artificial Sequence
  element 2
tccat

SEQ ID NO: 536 - DNA, 5 bp, Artificial Sequence
  Element 2
tccta

SEQ ID NO: 537 - DNA, 5 bp, Artificial Sequence
  Element 2
tctac

SEQ ID NO: 538 - DNA, 5 bp, Artificial Sequence
  Element 2
tctca

SEQ ID NO: 539 - DNA, 3 bp, Artificial Sequence
  Element 3
aag

SEQ ID NO: 540 - DNA, 3 bp, Artificial Sequence
  Element 3
ctc

SEQ ID NO: 541 - DNA, 3 bp, Artificial Sequence
  Element 3
ggt

SEQ ID NO: 542 - DNA, 3 bp, Artificial Sequence
  Element 3
tca

SEQ ID NO: 543 - DNA, 3 bp, Artificial Sequence
  Element 3
act

SEQ ID NO: 544 - DNA, 3 bp, Artificial Sequence
  Element 3
cga

SEQ ID NO: 545 - DNA, 3 bp, Artificial Sequence
  Element 3
gtg

SEQ ID NO: 546 - DNA, 3 bp, Artificial Sequence
  Element 3
tac

SEQ ID NO: 547 - DNA, 3 bp, Artificial Sequence
  Element 3
agc

SEQ ID NO: 548 - DNA, 3 bp, Artificial Sequence
  Element 3
ccg

SEQ ID NO: 549 - DNA, 3 bp, Artificial Sequence
  Element 3
gaa

SEQ ID NO: 550 - DNA, 3 bp, Artificial Sequence
  Element 3
ttt

SEQ ID NO: 551 - DNA, 3 bp, Artificial Sequence
  Element 3
ata

SEQ ID NO: 552 - DNA, 3 bp, Artificial Sequence
  Element 3
cat

SEQ ID NO: 553 - DNA, 3 bp, Artificial Sequence
  Element 3
gcc

SEQ ID NO: 554 - DNA, 3 bp, Artificial Sequence
  Element 3
tgg

SEQ ID NO: 555 - DNA, 12 bp, Artificial Sequence
  Element 4
acccacaccaaa

SEQ ID NO: 556 - DNA, 12 bp, Artificial Sequence
  Element 4
caaacacaaccc

SEQ ID NO: 557 - DNA, 12 bp, Artificial Sequence
  Element 4
gtgtgggttgtt

SEQ ID NO: 558 - DNA, 12 bp, Artificial Sequence
  Element 4
tgtgtttggtgg

SEQ ID NO: 559 - DNA, 12 bp, Artificial Sequence
  Element 4
tttggtgtgggt

SEQ ID NO: 560 - DNA, 12 bp, Artificial Sequence
  Element 4
gggttgtgtttg

SEQ ID NO: 561 - DNA, 12 bp, Artificial Sequence
  Element 4
aacaacccacac

SEQ ID NO: 562 - DNA, 12 bp, Artificial Sequence
  Element 4
ccaccaaacaca